European Patent Application EP 4 491 235 A2, published January 15, 2025. Title: Primary NK CAR Constructs and Methods. Applicant: ImmunityBio, Inc. Application EP. The sequence listing filed with the application follows.

SEQUENCE LISTING (4 sequences)

SEQ ID NO: 1 - DNA, 7584 bp, synthetic construct
  misc_feature 1..7584: note = XL53
  source 1..7584: mol_type = other DNA
agctgccttctgcggggcttgccttctggccatgcccttcttctctcccttgcacctgtacctcttggtctttgaataaagcctgagtaggaagaaaaaaaaaaaaaaaaaaaaaagcaggtggcggccgcaggtaagccagcccaggcctcgccctccagctcaaggcgggacaggtgccctagagtagcctgcatccagggacaggccccagccgggtgctgacacgtccacctccatctcttcctcaggtctgcccgggtggcatccctgtgacccctccccagtgcctctcctggtcgtggaaggtgctactccagtgcccaccagccttgtcctaataaaattaagttgcatcattttgtttgactaggtgtccttgtataatattatggggtggaggcgggtggtatggagcaaggggcccaagttaacttgtttattgcagcttataatggttacaaataaagcaatagcatcacaaatttcacaaataaagcatttttttcactgcattctagttgtggtttgtccaaactcatcaatgtatcttatcatgtctggatccgcttcaggcaccgggcttgcgggtcatgcaccaggtgcgcggtccttcgggcacctcgacgtcggcggtgacggtgaagccgagccgctcgtagaaggggaggttgcggggcgcggaggtctccaggaaggcgggcaccccggcgcgctcggccgcctccactccggggagcacgacggcgctgcccagacccttgccctggtggtcgggcgagacgccgacggtggccaggaaccacgcgggctccttgggccggtgcggcgccaggaggccttccatctgttgctgcgcggccagcctggaaccgctcaactcggccatgcgcgggccgatctcggcgaacaccgcccccgcttcgacgctctccggcgtggtccagaccgccaccgcggcgccgtcgtccgcgacccacaccttgccgatgtcgagcccgacgcgcgtgaggaagagttcttgcagctcggtgacccgctcgatgtggcggtccgggtcgacggtgtggcgcgtggcggggtagtcggcgaacgcggcggcgagggtgcgtacggcccgggggacgtcgtcgcgggtggcgaggcgcaccgtgggcttgtactcggtcatggtggcctgcagagtcgctctgtgttcgaggccacacgcgtcaccttaatatgcgaagtggacctgggaccgcgccgccccgactgcatctgcgtgttttcgccaatgacaagacgctgggcggggtttgtgtcatcatagaactaaagacatgcaaatatatttcttccggggacaccgccagcaaacgcgagcaacgggccacggggatgaagcagctgcgccactccctgaagatccatcgtctcctaacaagttacatcactcctgcccttcctcaccctcatctccatcacctccttcatctccgtcatctccgtcatcaccctccgcggcagccccttccaccataggtggaaaccagggaggcaaatctactccatcgtcaaagctgcacacagtcaccctgatattgcaggtaggagcgggctttgtcataacaaggtccttaatcgcatccttcaaaacctcagcaaatatatgagtttgtaaaaagaccatgaaataacagacaatggactcccttagcgggccaggttgtgggccgggtccaggggccattccaaaggggagacgactcaatggtgtaagacgacattgtggaatagcaagggcagttcctcgccttaggttgtaaagggaggtcttactacctccatatacgaacacaccggcgacccaagttccttcgtcggtagtcctttctacgtgactcctagccaggagagctcttaaaccttctgcaatgttctcaaatttcgggttggaacctccttgaccacgatgctttccaaaccaccctccttttttgcgcctgcctccatcaccctgacccccgctgcgcgggggcacgtcaggctcaccatctgggccgccttcttggtggtattcaaaataatcggcttcccctacagggtggaaaaatggccttctacctggagggggcctgcgcggtggagacccggatgatgatgactgactactgggactcctgggcctcttttctccacgtccacgacctctccccctggctctttcacgacttccccccctggctctttcacgtcctctaccccggcggcctccactacctcctcgaccccggcctccactacctcctcgaccccggcctccactgcctcctcgaccccggcctccacctcctgctcctgcccctcccgctcctgctcctgctcctgttccaccgtgggtccctttgcagccaatgcaacttggacgtttttggggtctccggacaccatctctatgtcttggccctgatcctgagccgcccggggctcctggtcttccgcctcctcgtcctcgtcctcttccccgtcctcgtccatgtgccatgatggcggcctgcagctgtgttcgaggccgcgcgtgtcaccttaatatgcgaagtggacctgggaccgcgccgccccgactgcatctgcgtgttcgagttcgccaatgacaagacgctgggcggggagatcccccttattaaccctaaacgggtagcatatgcttcccgggtagtagtatatactatccagactaaccctaattcaatagcatatgttacccaacgggaagcatatgctatcgaattagggttagtaaaagggtcctaaggaacagcgatctggatagcatatgctatcctaatctatatctgggtagcatatgctatcctaatctatatctgggtagcataggctatcctaatctatatctgggtagcatatgctatcctaatctatatctgggtagtatatgctatcctaatttatatctgggtagcataggctatcctaatctatatctgggtagcatatgctatcctatcctcatgcatatacagtcagcatatgatacccagtagtagagtgggagtgctatcctttgcatagcccatcccgcccctaactccgcccagttccgcccattctccgcctcatggctgactaattttttaggaggcttttttggaggcctaggcttttgcaaaaagctaattcggcgtaatctgctgcttgcaaacaaaaaaaccaccgctaccagcggtggtttgtttgccggatcaagagctaccaactctttttccgaaggtaactggcttcagcagagcgcagataccaaatactgtccttctagtgtagccgtagttaggccaccacttcaagaactctgtagcaccgcctacatacctcgctctgctgaagccagttaccagtggctgctgccagtggcgataagtcgtgtcttaccgggttggactcaagagatagttaccggataaggcgcagcggtcgggctgaacggggggttcgtgcacacagcccagcttggagcgaacgacctacaccgaactgagatacctacagcgtgagctatgagaaagcgccacgcttcccgaagggagaaaggcggacaggtatccggtaagcggcagggtcggaacaggagagcgcacgagggagcttccagggggaaacgcctggtatctttatagtcctgtcgggtttcgccacctctgacttgagcgtcgatttttgtgatgctcgtcaggggggcggagcctatggaaaaacgccagcaacgcaagctagagtttaaacttgacagatgagacaataaccctgataaatgcttcaataatattgaaaaaggaaaagtatgagtattcaacatttccgtgtcgcccttattcccttttttgcggcattttgccttcctgtttttgctcacccagaaacgctggtgaaagtaaaagatgcagaagatcacttgggtgcgcgagtgggttacatcgaactggatctcaacagcggtaagatccttgagagttttcgccccgaagaacgtttcccaatgatgagcacttttaaagttctgctatgtggcgcggtattatcccgtattgatgccgggcaagagcaactcggtcgccgcatacactattctcagaatgacttggttgaatactcaccagtcacagaaaagcatcttacggatggcatgacagtaagagaattatgcagtgctgccataaccatgagtgataacactgcggccaacttacttctgacaactatcggaggaccgaaggagctaaccgcttttttgcacaacatgggggatcatgtaactcgccttgatcgttgggaaccggagctgaatgaagccataccaaacgacgagcgtgacaccacgatgcctgtagcaatggcaacaacgttgcgaaaactattaactggcgaactacttactctagcttcccggcaacaactaatagactggatggaggcggataaagttgcaggaccacttctgcgctcggcacttccggctggctggtttattgctgataaatcaggagccggtgagcgtgggtcacgcggtatcattgcagcactggggccggatggtaagccctcccgtatcgtagttatctacactacggggagtcaggcaactatggatgaacgaaatagacagatcgctgagataggtgcctcactgattaagcattggtaaggataaatttctggtaaggaggacacgtatggaagtgggcaagttggggaagccgtatccgttgctgaatctggcatatgtgggagtataagacgcgcagcgtcgcatcaggcatttttttctgcgccaatgcaaaaaggccatccgtcaggatggcctttcggcataactagtgaggctccggtgcccgtcagtgggcagagcgcacatcgcccacagtccccgagaagttggggggaggggtcggcaattgaaccggtgcctagagaaggtggcgcggggtaaactgggaaagtgatgtcgtgtactggctccgcctttttcccgagggtgggggagaaccgtatataagtgcagtagtcgccgtgaacgttctttttcgcaacgggtttgccgccagaacacaggtaagtgccgtgtgtggttcccgcgggcctggcctctttacgggttatggcccttgcgtgccttgaattacttccacctggctgcagtacgtgattcttgatcccgagcttcgggttggaagtgggtgggagagttcgaggccttgcgcttaaggagccccttcgcctcgtgcttgagttgaggcctggcctgggcgctggggccgccgcgtgcgaatctggtggcaccttcgcgcctgtctcgctgctttcgataagtctctagccatttaaaatttttgatgacctgctgcgacgctttttttctggcaagatagtcttgtaaatgcgggccaagacgatctgcacactggtatttcggtttttggggccgcgggcggcgacggggcccgtgcgtcccagcgcacatgttcggcgaggcggggcctgcgagcgcggccaccgagaatcggacgggggtagtctcaagctggccggcctgctctggtgcctggcctcgcgccgccgtgtatcgccccgccctgggcggcaaggctggcccggtcggcaccagttgcgtgagcggaaagatggccgcttcccggccctgctgcagggagctcaaaatggaggacgcggcgctcgggagagcgggcgggtgagtcacccacacaaaggaaaagggcctttccgtcctcagccgtcgcttcatgtgactccacggagtaccgggcgccgtccaggcacctcgattagttctcgagcttttggagtacgtcgtctttaggttggggggaggggttttatgcgatggagtttccccacactgagtgggtggagactgaagttaggccagcttggcacttgatgtaattctccttggaatttgccctttttgagtttggatcttggttcattctcaagcctcagacagtggttcaaagtttttttcttccatttcaggtgtcgtgaaaagctttaatacgactcactatagggaaataagagagaaaagaagagtaagaagaaatataagagccaccatgtggtttcttactacattgctgttgtgggtcccggtggacggtaacatccagatgacccagtctccatcttctgtgtctgcatctgtaggagacagagtcaccatcacttgtcgggcgagtcaggatattagccgctggttagcctggtatcagcagaaaccagggaaagcccctaaactcctgatctatgctgcatccagtttgcaaagtggggtcccatcgaggttcagcggcagtggatctgggacagatttcgctctcactatcagcagcctgcagcctgaagattttgcaacttactattgtcaacaggctgacagtcgtttctcgatcaccttcggccaagggacacgactggagattaaaggcggcggaggaagcggaggcggaggatctgggggcggaggctctggcggagggggatctgaggtgcagctggtgcagtctgggggaggcttggtacagcctggggggtccctgagactctcctgtgcagcctctggattcaccttcagtagctatagcatgaactgggtccgccaggctccagggaaggggctggagtgggtttcatacattagtagtagtagtagtaccatacagtacgcagactctgtgaagggccgattcaccatctccagagacaatgccaagaactcactgtatctgcaaatgaacagcctgagagacgaggacacggctgtgtattactgtgcgagaggggactactactacggtatggacgtctggggccaagggaccacggtcaccgtgagctcaattgaagttatgtatcctcctccttacctagacaatgagaagagcaatggaaccattatccatgtgaaagggaaacacctttgtccaagtcccctatttcccggaccttctaagcccttttgggtgctggtggtggttggtggagtcctggcttgctatagcttgctagtaacagtggcctttattattttctgggtgaggagtaagaggagcaggctcctgcacagtgactacatgaacatgactccccgccgccccgggcccacccgcaagcattaccagccctatgccccaccacgcgacttcgcagcctatcgctccagagtgaagttcagcaggagcgcagacgcccccgcgtaccagcagggccagaaccagctctataacgagctcaatctaggacgaagagaggagtacgatgttttggacaagagacgtggccgggaccctgagatggggggaaagccgcagagaaggaagaaccctcaggaaggcctgtacaatgaactgcagaaagataagatggcggaggcctacagtgagattgggatgaaaggcgagcgccggaggggcaaggggcacgatggcctttaccagggtctcagtacagccaccaaggacacctacgacgcccttcacatgcaggccctgccccctcgctgattaatta

SEQ ID NO: 2 - DNA, 7709 bp, synthetic construct
  misc_feature 1..7709: note = XL53-150A
  source 1..7709: mol_type = other DNA
tcaaggcgggacaggtgccctagagtagcctgcatccagggacaggccccagccgggtgctgacacgtccacctccatctcttcctcaggtctgcccgggtggcatccctgtgacccctccccagtgcctctcctggtcgtggaaggtgctactccagtgcccaccagccttgtcctaataaaattaagttgcatcattttgtttgactaggtgtccttgtataatattatggggtggaggcgggtggtatggagcaaggggcccaagttaacttgtttattgcagcttataatggttacaaataaagcaatagcatcacaaatttcacaaataaagcatttttttcactgcattctagttgtggtttgtccaaactcatcaatgtatcttatcatgtctggatccgcttcaggcaccgggcttgcgggtcatgcaccaggtgcgcggtccttcgggcacctcgacgtcggcggtgacggtgaagccgagccgctcgtagaaggggaggttgcggggcgcggaggtctccaggaaggcgggcaccccggcgcgctcggccgcctccactccggggagcacgacggcgctgcccagacccttgccctggtggtcgggcgagacgccgacggtggccaggaaccacgcgggctccttgggccggtgcggcgccaggaggccttccatctgttgctgcgcggccagcctggaaccgctcaactcggccatgcgcgggccgatctcggcgaacaccgcccccgcttcgacgctctccggcgtggtccagaccgccaccgcggcgccgtcgtccgcgacccacaccttgccgatgtcgagcccgacgcgcgtgaggaagagttcttgcagctcggtgacccgctcgatgtggcggtccgggtcgacggtgtggcgcgtggcggggtagtcggcgaacgcggcggcgagggtgcgtacggcccgggggacgtcgtcgcgggtggcgaggcgcaccgtgggcttgtactcggtcatggtggcctgcagagtcgctctgtgttcgaggccacacgcgtcaccttaatatgcgaagtggacctgggaccgcgccgccccgactgcatctgcgtgttttcgccaatgacaagacgctgggcggggtttgtgtcatcatagaactaaagacatgcaaatatatttcttccggggacaccgccagcaaacgcgagcaacgggccacggggatgaagcagctgcgccactccctgaagatccatcgtctcctaacaagttacatcactcctgcccttcctcaccctcatctccatcacctccttcatctccgtcatctccgtcatcaccctccgcggcagccccttccaccataggtggaaaccagggaggcaaatctactccatcgtcaaagctgcacacagtcaccctgatattgcaggtaggagcgggctttgtcataacaaggtccttaatcgcatccttcaaaacctcagcaaatatatgagtttgtaaaaagaccatgaaataacagacaatggactcccttagcgggccaggttgtgggccgggtccaggggccattccaaaggggagacgactcaatggtgtaagacgacattgtggaatagcaagggcagttcctcgccttaggttgtaaagggaggtcttactacctccatatacgaacacaccggcgacccaagttccttcgtcggtagtcctttctacgtgactcctagccaggagagctcttaaaccttctgcaatgttctcaaatttcgggttggaacctccttgaccacgatgctttccaaaccaccctccttttttgcgcctgcctccatcaccctgacccccgctgcgcgggggcacgtcaggctcaccatctgggccgccttcttggtggtattcaaaataatcggcttcccctacagggtggaaaaatggccttctacctggagggggcctgcgcggtggagacccggatgatgatgactgactactgggactcctgggcctcttttctccacgtccacgacctctccccctggctctttcacgacttccccccctggctctttcacgtcctctaccccggcggcctccactacctcctcgaccccggcctccactacctcctcgaccccggcctccactgcctcctcgaccccggcctccacctcctgctcctgcccctcccgctcctgctcctgctcctgttccaccgtgggtccctttgcagccaatgcaacttggacgtttttggggtctccggacaccatctctatgtcttggccctgatcctgagccgcccggggctcctggtcttccgcctcctcgtcctcgtcctcttccccgtcctcgtccatgtgccatgatggcggcctgcagctgtgttcgaggccgcgcgtgtcaccttaatatgcgaagtggacctgggaccgcgccgccccgactgcatctgcgtgttcgagttcgccaatgacaagacgctgggcggggagatcccccttattaaccctaaacgggtagcatatgcttcccgggtagtagtatatactatccagactaaccctaattcaatagcatatgttacccaacgggaagcatatgctatcgaattagggttagtaaaagggtcctaaggaacagcgatctggatagcatatgctatcctaatctatatctgggtagcatatgctatcctaatctatatctgggtagcataggctatcctaatctatatctgggtagcatatgctatcctaatctatatctgggtagtatatgctatcctaatttatatctgggtagcataggctatcctaatctatatctgggtagcatatgctatcctatcctcatgcatatacagtcagcatatgatacccagtagtagagtgggagtgctatcctttgcatagcccatcccgcccctaactccgcccagttccgcccattctccgcctcatggctgactaattttttaggaggcttttttggaggcctaggcttttgcaaaaagctaattcggcgtaatctgctgcttgcaaacaaaaaaaccaccgctaccagcggtggtttgtttgccggatcaagagctaccaactctttttccgaaggtaactggcttcagcagagcgcagataccaaatactgtccttctagtgtagccgtagttaggccaccacttcaagaactctgtagcaccgcctacatacctcgctctgctgaagccagttaccagtggctgctgccagtggcgataagtcgtgtcttaccgggttggactcaagagatagttaccggataaggcgcagcggtcgggctgaacggggggttcgtgcacacagcccagcttggagcgaacgacctacaccgaactgagatacctacagcgtgagctatgagaaagcgccacgcttcccgaagggagaaaggcggacaggtatccggtaagcggcagggtcggaacaggagagcgcacgagggagcttccagggggaaacgcctggtatctttatagtcctgtcgggtttcgccacctctgacttgagcgtcgatttttgtgatgctcgtcaggggggcggagcctatggaaaaacgccagcaacgcaagctagagtttaaacttgacagatgagacaataaccctgataaatgcttcaataatattgaaaaaggaaaagtatgagtattcaacatttccgtgtcgcccttattcccttttttgcggcattttgccttcctgtttttgctcacccagaaacgctggtgaaagtaaaagatgcagaagatcacttgggtgcgcgagtgggttacatcgaactggatctcaacagcggtaagatccttgagagttttcgccccgaagaacgtttcccaatgatgagcacttttaaagttctgctatgtggcgcggtattatcccgtattgatgccgggcaagagcaactcggtcgccgcatacactattctcagaatgacttggttgaatactcaccagtcacagaaaagcatcttacggatggcatgacagtaagagaattatgcagtgctgccataaccatgagtgataacactgcggccaacttacttctgacaactatcggaggaccgaaggagctaaccgcttttttgcacaacatgggggatcatgtaactcgccttgatcgttgggaaccggagctgaatgaagccataccaaacgacgagcgtgacaccacgatgcctgtagcaatggcaacaacgttgcgaaaactattaactggcgaactacttactctagcttcccggcaacaactaatagactggatggaggcggataaagttgcaggaccacttctgcgctcggcacttccggctggctggtttattgctgataaatcaggagccggtgagcgtgggtcacgcggtatcattgcagcactggggccggatggtaagccctcccgtatcgtagttatctacactacggggagtcaggcaactatggatgaacgaaatagacagatcgctgagataggtgcctcactgattaagcattggtaaggataaatttctggtaaggaggacacgtatggaagtgggcaagttggggaagccgtatccgttgctgaatctggcatatgtgggagtataagacgcgcagcgtcgcatcaggcatttttttctgcgccaatgcaaaaaggccatccgtcaggatggcctttcggcataactagtgaggctccggtgcccgtcagtgggcagagcgcacatcgcccacagtccccgagaagttggggggaggggtcggcaattgaaccggtgcctagagaaggtggcgcggggtaaactgggaaagtgatgtcgtgtactggctccgcctttttcccgagggtgggggagaaccgtatataagtgcagtagtcgccgtgaacgttctttttcgcaacgggtttgccgccagaacacaggtaagtgccgtgtgtggttcccgcgggcctggcctctttacgggttatggcccttgcgtgccttgaattacttccacctggctgcagtacgtgattcttgatcccgagcttcgggttggaagtgggtgggagagttcgaggccttgcgcttaaggagccccttcgcctcgtgcttgagttgaggcctggcctgggcgctggggccgccgcgtgcgaatctggtggcaccttcgcgcctgtctcgctgctttcgataagtctctagccatttaaaatttttgatgacctgctgcgacgctttttttctggcaagatagtcttgtaaatgcgggccaagacgatctgcacactggtatttcggtttttggggccgcgggcggcgacggggcccgtgcgtcccagcgcacatgttcggcgaggcggggcctgcgagcgcggccaccgagaatcggacgggggtagtctcaagctggccggcctgctctggtgcctggcctcgcgccgccgtgtatcgccccgccctgggcggcaaggctggcccggtcggcaccagttgcgtgagcggaaagatggccgcttcccggccctgctgcagggagctcaaaatggaggacgcggcgctcgggagagcgggcgggtgagtcacccacacaaaggaaaagggcctttccgtcctcagccgtcgcttcatgtgactccacggagtaccgggcgccgtccaggcacctcgattagttctcgagcttttggagtacgtcgtctttaggttggggggaggggttttatgcgatggagtttccccacactgagtgggtggagactgaagttaggccagcttggcacttgatgtaattctccttggaatttgccctttttgagtttggatcttggttcattctcaagcctcagacagtggttcaaagtttttttcttccatttcaggtgtcgtgaaaagctttaatacgactcactatagggaaataagagagaaaagaagagtaagaagaaatataagagccaccatgtggtttcttactacattgctgttgtgggtcccggtggacggtaacatccagatgacccagtctccatcttctgtgtctgcatctgtaggagacagagtcaccatcacttgtcgggcgagtcaggatattagccgctggttagcctggtatcagcagaaaccagggaaagcccctaaactcctgatctatgctgcatccagtttgcaaagtggggtcccatcgaggttcagcggcagtggatctgggacagatttcgctctcactatcagcagcctgcagcctgaagattttgcaacttactattgtcaacaggctgacagtcgtttctcgatcaccttcggccaagggacacgactggagattaaaggcggcggaggaagcggaggcggaggatctgggggcggaggctctggcggagggggatctgaggtgcagctggtgcagtctgggggaggcttggtacagcctggggggtccctgagactctcctgtgcagcctctggattcaccttcagtagctatagcatgaactgggtccgccaggctccagggaaggggctggagtgggtttcatacattagtagtagtagtagtaccatacagtacgcagactctgtgaagggccgattcaccatctccagagacaatgccaagaactcactgtatctgcaaatgaacagcctgagagacgaggacacggctgtgtattactgtgcgagaggggactactactacggtatggacgtctggggccaagggaccacggtcaccgtgagctcaattgaagttatgtatcctcctccttacctagacaatgagaagagtaatggaaccattatccatgtgaaagggaaacacctttgtccaagtcccctatttcccggaccttctaagcccttttgggtgctggtggtggttggtggagtcctggcttgctatagcttgctagtaacagtggcctttattattttctgggtgaggagtaagaggagcaggctcctgcacagtgactacatgaacatgactccccgccgccccgggcccacccgcaagcattaccagccctatgccccaccacgcgacttcgcagcctatcgctccagagtgaagttcagcaggagcgcagacgcccccgcgtaccagcagggccagaaccagctctataacgagctcaatctaggacgaagagaggagtacgatgttttggacaagagacgtggccgggaccctgagatggggggaaagccgcagagaaggaagaaccctcaggaaggcctgtacaatgaactgcagaaagataagatggcggaggcctacagtgagattgggatgaaaggcgagcgccggaggggcaaggggcacgatggcctttaccagggtctcagtacagccaccaaggacacctacgacgcccttcacatgcaggccctgccccctcgctgattaattaagctgccttctgcggggcttgccttctggccatgcccttcttctctcccttgcacctgtacctcttggtctttgaataaagcctgagtaggaagggtaccaaaaaaaaaaaaaaaaaaaaaaaaaaaaaaaaaaaaaaaaaaaaaaaaaaaaaaaaaaaaaaaaaaaaaaaaaaaaaaaaaaaaaaaaaaaaaaaaaaaaaaaaaaaaaaaaaaaaaaaaaaaaaaaaaaaaaaaaaaaaaaaaaaaaaagaagagctctaggctagcccaggcctcgccctccagc

SEQ ID NO: 3 - DNA, 7493 bp, synthetic construct
  misc_feature 1..7493: note = NKW29
  source 1..7493: mol_type = other DNA
aggctccggtgcccgtcagtgggcagagcgcacatcgcccacagtccccgagaagttggggggaggggtcggcaattgaaccggtgcctagagaaggtggcgcggggtaaactgggaaagtgatgtcgtgtactggctccgcctttttcccgagggtgggggagaaccgtatataagtgcagtagtcgccgtgaacgttctttttcgcaacgggtttgccgccagaacacaggtaagtgccgtgtgtggttcccgcgggcctggcctctttacgggttatggcccttgcgtgccttgaattacttccacctggctgcagtacgtgattcttgatcccgagcttcgggttggaagtgggtgggagagttcgaggccttgcgcttaaggagccccttcgcctcgtgcttgagttgaggcctggcctgggcgctggggccgccgcgtgcgaatctggtggcaccttcgcgcctgtctcgctgctttcgataagtctctagccatttaaaatttttgatgacctgctgcgacgctttttttctggcaagatagtcttgtaaatgcgggccaagacgatctgcacactggtatttcggtttttggggccgcgggcggcgacggggcccgtgcgtcccagcgcacatgttcggcgaggcggggcctgcgagcgcggccaccgagaatcggacgggggtagtctcaagctggccggcctgctctggtgcctggcctcgcgccgccgtgtatcgccccgccctgggcggcaaggctggcccggtcggcaccagttgcgtgagcggaaagatggccgcttcccggccctgctgcagggagctcaaaatggaggacgcggcgctcgggagagcgggcgggtgagtcacccacacaaaggaaaagggcctttccgtcctcagccgtcgcttcatgtgactccacggagtaccgggcgccgtccaggcacctcgattagttctcgagcttttggagtacgtcgtctttaggttggggggaggggttttatgcgatggagtttccccacactgagtgggtggagactgaagttaggccagcttggcacttgatgtaattctccttggaatttgccctttttgagtttggatcttggttcattctcaagcctcagacagtggttcaaagtttttttcttccatttcaggtgtcgtgaaaagctttaatacgactcactatagggaaataagagagaaaagaagagtaagaagaaatataagagccaccatgtggtttcttactacattgctgttgtgggtcccggtggacggtaacatccagatgacccagtctccatcttctgtgtctgcatctgtaggagacagagtcaccatcacttgtcgggcgagtcaggatattagccgctggttagcctggtatcagcagaaaccagggaaagcccctaaactcctgatctatgctgcatccagtttgcaaagtggggtcccatcgaggttcagcggcagtggatctgggacagatttcgctctcactatcagcagcctgcagcctgaagattttgcaacttactattgtcaacaggctgacagtcgtttctcgatcaccttcggccaagggacacgactggagattaaaggcggcggaggaagcggaggcggaggatctgggggcggaggctctggcggagggggatctgaggtgcagctggtgcagtctgggggaggcttggtacagcctggggggtccctgagactctcctgtgcagcctctggattcaccttcagtagctatagcatgaactgggtccgccaggctccagggaaggggctggagtgggtttcatacattagtagtagtagtagtaccatacagtacgcagactctgtgaagggccgattcaccatctccagagacaatgccaagaactcactgtatctgcaaatgaacagcctgagagacgaggacacggctgtgtattactgtgcgagaggggactactactacggtatggacgtctggggccaagggaccacggtcaccgtgagctcaattgaagttatgtatcctcctccttacctagacaatgagaagagtaatggaaccattatccatgtgaaagggaaacacctttgtccaagtcccctatttcccggaccttctaagcccttttgggtgctggtggtggttggtggagtcctggcttgctatagcttgctagtaacagtggcctttattattttctgggtgaggagtaagaggagcaggctcctgcacagtgactacatgaacatgactccccgccgccccgggcccacccgcaagcattaccagccctatgccccaccacgcgacttcgcagcctatcgctccctgaagatccaggtccgaaaggccgccatcaccagctacgagaagtctgatggcgtgtacaccggcctgagcaccagaaaccaggaaacctacgagacactgaagcacgagaagcccccccagtgattaattaagctgccttctgcggggcttgccttctggccatgcccttcttctctcccttgcacctgtacctcttggtctttgaataaagcctgagtaggaagggtaccaaaaaaaaaaaaaaaaaaaaaaaaaaaaaaaaaaaaaaaaaaaaaaaaaaaaaaaaaaaaaaaaaaaaaaaaaaaaaaaaaaaaaaaaaaaaaaaaaaaaaaaaaaaaaaaaaaaaaaaaaaaaaaaaaaaaaaaaaaaaaaaaaaaaaagaagagctctaggctagcccaggcctcgccctccagctcaaggcgggacaggtgccctagagtagcctgcatccagggacaggccccagccgggtgctgacacgtccacctccatctcttcctcaggtctgcccgggtggcatccctgtgacccctccccagtgcctctcctggtcgtggaaggtgctactccagtgcccaccagccttgtcctaataaaattaagttgcatcattttgtttgactaggtgtccttgtataatattatggggtggaggcgggtggtatggagcaaggggcccaagttaacttgtttattgcagcttataatggttacaaataaagcaatagcatcacaaatttcacaaataaagcatttttttcactgcattctagttgtggtttgtccaaactcatcaatgtatcttatcatgtctggatccgcttcaggcaccgggcttgcgggtcatgcaccaggtgcgcggtccttcgggcacctcgacgtcggcggtgacggtgaagccgagccgctcgtagaaggggaggttgcggggcgcggaggtctccaggaaggcgggcaccccggcgcgctcggccgcctccactccggggagcacgacggcgctgcccagacccttgccctggtggtcgggcgagacgccgacggtggccaggaaccacgcgggctccttgggccggtgcggcgccaggaggccttccatctgttgctgcgcggccagcctggaaccgctcaactcggccatgcgcgggccgatctcggcgaacaccgcccccgcttcgacgctctccggcgtggtccagaccgccaccgcggcgccgtcgtccgcgacccacaccttgccgatgtcgagcccgacgcgcgtgaggaagagttcttgcagctcggtgacccgctcgatgtggcggtccgggtcgacggtgtggcgcgtggcggggtagtcggcgaacgcggcggcgagggtgcgtacggcccgggggacgtcgtcgcgggtggcgaggcgcaccgtgggcttgtactcggtcatggtggcctgcagagtcgctctgtgttcgaggccacacgcgtcaccttaatatgcgaagtggacctgggaccgcgccgccccgactgcatctgcgtgttttcgccaatgacaagacgctgggcggggtttgtgtcatcatagaactaaagacatgcaaatatatttcttccggggacaccgccagcaaacgcgagcaacgggccacggggatgaagcagctgcgccactccctgaagatccatcgtctcctaacaagttacatcactcctgcccttcctcaccctcatctccatcacctccttcatctccgtcatctccgtcatcaccctccgcggcagccccttccaccataggtggaaaccagggaggcaaatctactccatcgtcaaagctgcacacagtcaccctgatattgcaggtaggagcgggctttgtcataacaaggtccttaatcgcatccttcaaaacctcagcaaatatatgagtttgtaaaaagaccatgaaataacagacaatggactcccttagcgggccaggttgtgggccgggtccaggggccattccaaaggggagacgactcaatggtgtaagacgacattgtggaatagcaagggcagttcctcgccttaggttgtaaagggaggtcttactacctccatatacgaacacaccggcgacccaagttccttcgtcggtagtcctttctacgtgactcctagccaggagagctcttaaaccttctgcaatgttctcaaatttcgggttggaacctccttgaccacgatgctttccaaaccaccctccttttttgcgcctgcctccatcaccctgacccccgctgcgcgggggcacgtcaggctcaccatctgggccgccttcttggtggtattcaaaataatcggcttcccctacagggtggaaaaatggccttctacctggagggggcctgcgcggtggagacccggatgatgatgactgactactgggactcctgggcctcttttctccacgtccacgacctctccccctggctctttcacgacttccccccctggctctttcacgtcctctaccccggcggcctccactacctcctcgaccccggcctccactacctcctcgaccccggcctccactgcctcctcgaccccggcctccacctcctgctcctgcccctcccgctcctgctcctgctcctgttccaccgtgggtccctttgcagccaatgcaacttggacgtttttggggtctccggacaccatctctatgtcttggccctgatcctgagccgcccggggctcctggtcttccgcctcctcgtcctcgtcctcttccccgtcctcgtccatgtgccatgatggcggcctgcagctgtgttcgaggccgcgcgtgtcaccttaatatgcgaagtggacctgggaccgcgccgccccgactgcatctgcgtgttcgagttcgccaatgacaagacgctgggcggggagatcccccttattaaccctaaacgggtagcatatgcttcccgggtagtagtatatactatccagactaaccctaattcaatagcatatgttacccaacgggaagcatatgctatcgaattagggttagtaaaagggtcctaaggaacagcgatctggatagcatatgctatcctaatctatatctgggtagcatatgctatcctaatctatatctgggtagcataggctatcctaatctatatctgggtagcatatgctatcctaatctatatctgggtagtatatgctatcctaatttatatctgggtagcataggctatcctaatctatatctgggtagcatatgctatcctatcctcatgcatatacagtcagcatatgatacccagtagtagagtgggagtgctatcctttgcatagcccatcccgcccctaactccgcccagttccgcccattctccgcctcatggctgactaattttttaggaggcttttttggaggcctaggcttttgcaaaaagctaattcggcgtaatctgctgcttgcaaacaaaaaaaccaccgctaccagcggtggtttgtttgccggatcaagagctaccaactctttttccgaaggtaactggcttcagcagagcgcagataccaaatactgtccttctagtgtagccgtagttaggccaccacttcaagaactctgtagcaccgcctacatacctcgctctgctgaagccagttaccagtggctgctgccagtggcgataagtcgtgtcttaccgggttggactcaagagatagttaccggataaggcgcagcggtcgggctgaacggggggttcgtgcacacagcccagcttggagcgaacgacctacaccgaactgagatacctacagcgtgagctatgagaaagcgccacgcttcccgaagggagaaaggcggacaggtatccggtaagcggcagggtcggaacaggagagcgcacgagggagcttccagggggaaacgcctggtatctttatagtcctgtcgggtttcgccacctctgacttgagcgtcgatttttgtgatgctcgtcaggggggcggagcctatggaaaaacgccagcaacgcaagctagagtttaaacttgacagatgagacaataaccctgataaatgcttcaataatattgaaaaaggaaaagtatgagtattcaacatttccgtgtcgcccttattcccttttttgcggcattttgccttcctgtttttgctcacccagaaacgctggtgaaagtaaaagatgcagaagatcacttgggtgcgcgagtgggttacatcgaactggatctcaacagcggtaagatccttgagagttttcgccccgaagaacgtttcccaatgatgagcacttttaaagttctgctatgtggcgcggtattatcccgtattgatgccgggcaagagcaactcggtcgccgcatacactattctcagaatgacttggttgaatactcaccagtcacagaaaagcatcttacggatggcatgacagtaagagaattatgcagtgctgccataaccatgagtgataacactgcggccaacttacttctgacaactatcggaggaccgaaggagctaaccgcttttttgcacaacatgggggatcatgtaactcgccttgatcgttgggaaccggagctgaatgaagccataccaaacgacgagcgtgacaccacgatgcctgtagcaatggcaacaacgttgcgaaaactattaactggcgaactacttactctagcttcccggcaacaactaatagactggatggaggcggataaagttgcaggaccacttctgcgctcggcacttccggctggctggtttattgctgataaatcaggagccggtgagcgtgggtcacgcggtatcattgcagcactggggccggatggtaagccctcccgtatcgtagttatctacactacggggagtcaggcaactatggatgaacgaaatagacagatcgctgagataggtgcctcactgattaagcattggtaaggataaatttctggtaaggaggacacgtatggaagtgggcaagttggggaagccgtatccgttgctgaatctggcatatgtgggagtataagacgcgcagcgtcgcatcaggcatttttttctgcgccaatgcaaaaaggccatccgtcaggatggcctttcggcataactagtg

SEQ ID NO: 4 - DNA, 9496 bp, synthetic construct
  misc_feature 1..9496: note = XL53-Tri-cistronic
  source 1..9496: mol_type = other DNA
tgacagatgagacaataaccctgataaatgcttcaataatattgaaaaaggaaaagtatgagtattcaacatttccgtgtcgcccttattcccttttttgcggcattttgccttcctgtttttgctcacccagaaacgctggtgaaagtaaaagatgcagaagatcacttgggtgcgcgagtgggttacatcgaactggatctcaacagcggtaagatccttgagagttttcgccccgaagaacgtttcccaatgatgagcacttttaaagttctgctatgtggcgcggtattatcccgtattgatgccgggcaagagcaactcggtcgccgcatacactattctcagaatgacttggttgaatactcaccagtcacagaaaagcatcttacggatggcatgacagtaagagaattatgcagtgctgccataaccatgagtgataacactgcggccaacttacttctgacaactatcggaggaccgaaggagctaaccgcttttttgcacaacatgggggatcatgtaactcgccttgatcgttgggaaccggagctgaatgaagccataccaaacgacgagcgtgacaccacgatgcctgtagcaatggcaacaacgttgcgaaaactattaactggcgaactacttactctagcttcccggcaacaactaatagactggatggaggcggataaagttgcaggaccacttctgcgctcggcacttccggctggctggtttattgctgataaatcaggagccggtgagcgtgggtcacgcggtatcattgcagcactggggccggatggtaagccctcccgtatcgtagttatctacactacggggagtcaggcaactatggatgaacgaaatagacagatcgctgagataggtgcctcactgattaagcattggtaaggataaatttctggtaaggaggacacgtatggaagtgggcaagttggggaagccgtatccgttgctgaatctggcatatgtgggagtataagacgcgcagcgtcgcatcaggcatttttttctgcgccaatgcaaaaaggccatccgtcaggatggcctttcggcataactagtgaggctccggtgcccgtcagtgggcagagcgcacatcgcccacagtccccgagaagttggggggaggggtcggcaattgaaccggtgcctagagaaggtggcgcggggtaaactgggaaagtgatgtcgtgtactggctccgcctttttcccgagggtgggggagaaccgtatataagtgcagtagtcgccgtgaacgttctttttcgcaacgggtttgccgccagaacacaggtaagtgccgtgtgtggttcccgcgggcctggcctctttacgggttatggcccttgcgtgccttgaattacttccacctggctgcagtacgtgattcttgatcccgagcttcgggttggaagtgggtgggagagttcgaggccttgcgcttaaggagccccttcgcctcgtgcttgagttgaggcctggcctgggcgctggggccgccgcgtgcgaatctggtggcaccttcgcgcctgtctcgctgctttcgataagtctctagccatttaaaatttttgatgacctgctgcgacgctttttttctggcaagatagtcttgtaaatgcgggccaagacgatctgcacactggtatttcggtttttggggccgcgggcggcgacggggcccgtgcgtcccagcgcacatgttcggcgaggcggggcctgcgagcgcggccaccgagaatcggacgggggtagtctcaagctggccggcctgctctggtgcctggcctcgcgccgccgtgtatcgccccgccctgggcggcaaggctggcccggtcggcaccagttgcgtgagcggaaagatggccgcttcccggccctgctgcagggagctcaaaatggaggacgcggcgctcgggagagcgggcgggtgagtcacccacacaaaggaaaagggcctttccgtcctcagccgtcgcttcatgtgactccacggagtaccgggcgccgtccaggcacctcgattagttctcgagcttttggagtacgtcgtctttaggttggggggaggggttttatgcgatggagtttccccacactgagtgggtggagactgaagttaggccagcttggcacttgatgtaattctccttggaatttgccctttttgagtttggatcttggttcattctcaagcctcagacagtggttcaaagtttttttcttccatttcaggtgtcgtgaaaagctttaatacgactcactatagggaaataagagagaaaagaagagtaagaagaaatataagagccaccatgtggtttcttactacattgctgttgtgggtcccggtggacggtaacatccagatgacccagtctccatcttctgtgtctgcatctgtaggagacagagtcaccatcacttgtcgggcgagtcaggatattagccgctggttagcctggtatcagcagaaaccagggaaagcccctaaactcctgatctatgctgcatccagtttgcaaagtggggtcccatcgaggttcagcggcagtggatctgggacagatttcgctctcactatcagcagcctgcagcctgaagattttgcaacttactattgtcaacaggctgacagtcgtttctcgatcaccttcggccaagggacacgactggagattaaaggcggcggaggaagcggaggcggaggatctgggggcggaggctctggcggagggggatctgaggtgcagctggtgcagtctgggggaggcttggtacagcctggggggtccctgagactctcctgtgcagcctctggattcaccttcagtagctatagcatgaactgggtccgccaggctccagggaaggggctggagtgggtttcatacattagtagtagtagtagtaccatacagtacgcagactctgtgaagggccgattcaccatctccagagacaatgccaagaactcactgtatctgcaaatgaacagcctgagagacgaggacacggctgtgtattactgtgcgagaggggactactactacggtatggacgtctggggccaagggaccacggtcaccgtgagctcaattgaagttatgtatcctcctccttacctagacaatgagaagagcaatggaaccattatccatgtgaaagggaaacacctttgtccaagtcccctatttcccggaccttctaagcccttttgggtgctggtggtggttggtggagtcctggcttgctatagcttgctagtaacagtggcctttattattttctgggtgaggagtaagaggagcaggctcctgcacagtgactacatgaacatgactccccgccgccccgggcccacccgcaagcattaccagccctatgccccaccacgcgacttcgcagcctatcgctccagagtgaagttcagcaggagcgcagacgcccccgcgtaccagcagggccagaaccagctctataacgagctcaatctaggacgaagagaggagtacgatgttttggacaagagacgtggccgggaccctgagatggggggaaagccgcagagaaggaagaaccctcaggaaggcctgtacaatgaactgcagaaagataagatggcggaggcctacagtgagattgggatgaaaggcgagcgccggaggggcaaggggcacgatggcctttaccagggtctcagtacagccaccaaggacacctacgacgcccttcacatgcaggccctgccccctcgcggatctggagctactaacttcagcctgctgaagcaggctggagacgtggaggagaaccctggacctatgtggcagctgctgctgcctacagctctcctgctgctggtgtccgccggcatgagaaccgaggatctgcctaaggccgtggtgttcctggaaccccagtggtacagagtgctggaaaaggacagcgtgaccctgaagtgccagggcgcctacagccccgaggacaatagcacccagtggttccacaacgagagcctgatcagcagccaggccagcagctacttcatcgacgccgccaccgtggacgacagcggcgagtatagatgccagaccaacctgagcaccctgagcgaccccgtgcagctggaagtgcacatcggatggctgctgctgcaggcccccagatgggtgttcaaagaagaggaccccatccacctgagatgccactcttggaagaacaccgccctgcacaaagtgacctacctgcagaacggcaagggcagaaagtacttccaccacaacagcgacttctacatccccaaggccaccctgaaggactccggctcctacttctgcagaggcctcgtgggcagcaagaacgtgtccagcgagacagtgaacatcaccatcacccagggcctggccgtgtctaccatcagcagctttttcccacccggctaccaggtgtccttctgcctcgtgatggtgctgctgttcgccgtggacaccggcctgtacttcagcgtgaaaacaaacatcagaagcagcacccgggactggaaggaccacaagttcaagtggcggaaggacccccaggacaagtgaaattccgcccctctcccccccccccctctccctcccccccccctaacgttactggccgaagccgcttggaataaggccggtgtgcgtttgtctatatgttattttccaccatattgccgtcttttggcaatgtgagggcccggaaacctggccctgtcttcttgacgagcattcctaggggtctttcccctctcgccaaaggaatgcaaggtctgttgaatgtcgtgaaggaagcagttcctctggaagcttcttgaagacaaacaacgtctgtagcgaccctttgcaggcagcggaaccccccacctggcgacaggtgcctctgcggccaaaagccacgtgtataagatacacctgcaaaggcggcacaaccccagtgccacgttgtgagttggatagttgtggaaagagtcaaatggctctcctcaagcgtattcaacaaggggctgaaggatgcccagaaggtaccccattgtatgggatctgatctggggcctcggtgcacatgctttacatgtgtttagtcgaggttaaaaaaacgtctaggccccccgaaccacggggacgtggttttcctttgaaaaacacgataaccgccaccatgtaccggatgcagctgctgagctgtatcgccctgtctctggccctcgtgaccaacagcgcccctaccagcagcagcaccaagaaaacccagctgcagctggaacatctgctgctggacctgcagatgatcctgaacggcatcaacaactacaagaaccccaagctgacccggatgctgaccttcaagttctacatgcccaagaaggccaccgaactgaaacatctgcagtgcctggaagaggaactgaagcccctggaagaagtgctgaacctggcccagagcaagaacttccacctgaggcccagggacctgatcagcaacatcaacgtgatcgtgctggaactgaaaggcagcgagacaaccttcatgtgcgagtacgccgacgagacagctaccatcgtggaatttctgaaccggtggatcaccttctgccagagcatcatcagcaccctgaccggctccgagaaggacgagctgtgattaattaagctgccttctgcggggcttgccttctggccatgcccttcttctctcccttgcacctgtacctcttggtctttgaataaagcctgagtaggaagaaaaaaaaaaaaaaaaaaaaaagcaggtggcggccgcaggtaagccagcccaggcctcgccctccagctcaaggcgggacaggtgccctagagtagcctgcatccagggacaggccccagccgggtgctgacacgtccacctccatctcttcctcaggtctgcccgggtggcatccctgtgacccctccccagtgcctctcctggtcgtggaaggtgctactccagtgcccaccagccttgtcctaataaaattaagttgcatcattttgtttgactaggtgtccttgtataatattatggggtggaggcgggtggtatggagcaaggggcccaagttaacttgtttattgcagcttataatggttacaaataaagcaatagcatcacaaatttcacaaataaagcatttttttcactgcattctagttgtggtttgtccaaactcatcaatgtatcttatcatgtctggatccgcttcaggcaccgggcttgcgggtcatgcaccaggtgcgcggtccttcgggcacctcgacgtcggcggtgacggtgaagccgagccgctcgtagaaggggaggttgcggggcgcggaggtctccaggaaggcgggcaccccggcgcgctcggccgcctccactccggggagcacgacggcgctgcccagacccttgccctggtggtcgggcgagacgccgacggtggccaggaaccacgcgggctccttgggccggtgcggcgccaggaggccttccatctgttgctgcgcggccagcctggaaccgctcaactcggccatgcgcgggccgatctcggcgaacaccgcccccgcttcgacgctctccggcgtggtccagaccgccaccgcggcgccgtcgtccgcgacccacaccttgccgatgtcgagcccgacgcgcgtgaggaagagttcttgcagctcggtgacccgctcgatgtggcggtccgggtcgacggtgtggcgcgtggcggggtagtcggcgaacgcggcggcgagggtgcgtacggcccgggggacgtcgtcgcgggtggcgaggcgcaccgtgggcttgtactcggtcatggtggcctgcagagtcgctctgtgttcgaggccacacgcgtcaccttaatatgcgaagtggacctgggaccgcgccgccccgactgcatctgcgtgttttcgccaatgacaagacgctgggcggggtttgtgtcatcatagaactaaagacatgcaaatatatttcttccggggacaccgccagcaaacgcgagcaacgggccacggggatgaagcagctgcgccactccctgaagatccatcgtctcctaacaagttacatcactcctgcccttcctcaccctcatctccatcacctccttcatctccgtcatctccgtcatcaccctccgcggcagccccttccaccataggtggaaaccagggaggcaaatctactccatcgtcaaagctgcacacagtcaccctgatattgcaggtaggagcgggctttgtcataacaaggtccttaatcgcatccttcaaaacctcagcaaatatatgagtttgtaaaaagaccatgaaataacagacaatggactcccttagcgggccaggttgtgggccgggtccaggggccattccaaaggggagacgactcaatggtgtaagacgacattgtggaatagcaagggcagttcctcgccttaggttgtaaagggaggtcttactacctccatatacgaacacaccggcgacccaagttccttcgtcggtagtcctttctacgtgactcctagccaggagagctcttaaaccttctgcaatgttctcaaatttcgggttggaacctccttgaccacgatgctttccaaaccaccctccttttttgcgcctgcctccatcaccctgacccccgctgcgcgggggcacgtcaggctcaccatctgggccgccttcttggtggtattcaaaataatcggcttcccctacagggtggaaaaatggccttctacctggagggggcctgcgcggtggagacccggatgatgatgactgactactgggactcctgggcctcttttctccacgtccacgacctctccccctggctctttcacgacttccccccctggctctttcacgtcctctaccccggcggcctccactacctcctcgaccccggcctccactacctcctcgaccccggcctccactgcctcctcgaccccggcctccacctcctgctcctgcccctcccgctcctgctcctgctcctgttccaccgtgggtccctttgcagccaatgcaacttggacgtttttggggtctccggacaccatctctatgtcttggccctgatcctgagccgcccggggctcctggtcttccgcctcctcgtcctcgtcctcttccccgtcctcgtccatgtgccatgatggcggcctgcagctgtgttcgaggccgcgcgtgtcaccttaatatgcgaagtggacctgggaccgcgccgccccgactgcatctgcgtgttcgagttcgccaatgacaagacgctgggcggggagatcccccttattaaccctaaacgggtagcatatgcttcccgggtagtagtatatactatccagactaaccctaattcaatagcatatgttacccaacgggaagcatatgctatcgaattagggttagtaaaagggtcctaaggaacagcgatctggatagcatatgctatcctaatctatatctgggtagcatatgctatcctaatctatatctgggtagcataggctatcctaatctatatctgggtagcatatgctatcctaatctatatctgggtagtatatgctatcctaatttatatctgggtagcataggctatcctaatctatatctgggtagcatatgctatcctatcctcatgcatatacagtcagcatatgatacccagtagtagagtgggagtgctatcctttgcatagcccatcccgcccctaactccgcccagttccgcccattctccgcctcatggctgactaattttttaggaggcttttttggaggcctaggcttttgcaaaaagctaattcggcgtaatctgctgcttgcaaacaaaaaaaccaccgctaccagcggtggtttgtttgccggatcaagagctaccaactctttttccgaaggtaactggcttcagcagagcgcagataccaaatactgtccttctagtgtagccgtagttaggccaccacttcaagaactctgtagcaccgcctacatacctcgctctgctgaagccagttaccagtggctgctgccagtggcgataagtcgtgtcttaccgggttggactcaagagatagttaccggataaggcgcagcggtcgggctgaacggggggttcgtgcacacagcccagcttggagcgaacgacctacaccgaactgagatacctacagcgtgagctatgagaaagcgccacgcttcccgaagggagaaaggcggacaggtatccggtaagcggcagggtcggaacaggagagcgcacgagggagcttccagggggaaacgcctggtatctttatagtcctgtcgggtttcgccacctctgacttgagcgtcgatttttgtgatgctcgtcaggggggcggagcctatggaaaaacgccagcaacgcaagctagagtttaaact